European Patent Application EP 4 696 714 A1, published February 18, 2026. Title: PREPARATION METHOD FOR NANOBODY TARGETING TISSUE FACTOR AND CONJUGATE AND USE THEREOF. Applicant: FUDAN UNIVERSITY. The sequence listing filed with the application follows.

SEQUENCE LISTING (35 sequences)

SEQ ID NO: 1 - protein, 8 aa, synthetic construct
  source 1..8: note = 4-A02 CDR1
ETISSTYI

SEQ ID NO: 2 - protein, 8 aa, synthetic construct
  source 1..8: note = 4-A02 CDR2
ISGDGVTH

SEQ ID NO: 3 - protein, 8 aa, synthetic construct
  source 1..8: note = 4-A02 CDR3
YAAGRWNH

SEQ ID NO: 4 - protein, 114 aa, synthetic construct
  source 1..114: note = 4-A02 VH
QVQLVESGGGLVQPGGSLSLSCTASETISSTYIMGWHRRSPGKERELVAVISGDGVTHYADFVKGRFVISRDNAKNAVYLKMNFLTPEDTAVYYCYAAGRWNHWGQGTQVTVSS

SEQ ID NO: 5 - protein, 8 aa, synthetic construct
  source 1..8: note = F1-A01 CDR1
GRAFSAYA

SEQ ID NO: 6 - protein, 8 aa, synthetic construct
  source 1..8: note = F1-A01 CDR2
ISWSGGST

SEQ ID NO: 7 - protein, 22 aa, synthetic construct
  source 1..22: note = F1-A01 CDR3
NADSLLSLLDGSRGGPGTDSGS

SEQ ID NO: 8 - protein, 129 aa, synthetic construct
  source 1..129: note = F1-A01 VH
EVQLVESGGGLVQAGGSLRLSCAASGRAFSAYAMGWFRQAPGKEREFVAAISWSGGSTYYADSVRGRFTISRDNTKNTVYLQMNSLKPEDTAVYYCNADSLLSLLDGSRGGPGTDSGSWGQGTQVTVSS

SEQ ID NO: 9 - protein, 8 aa, synthetic construct
  source 1..8: note = 4-C08 CDR1
GFSLSSYD

SEQ ID NO: 10 - protein, 8 aa, synthetic construct
  source 1..8: note = 4-C08 CDR2
IHSSGGYP

SEQ ID NO: 11 - protein, 12 aa, synthetic construct
  source 1..12: note = 4-C08 CDR3
NLPPSRRWYKDY

SEQ ID NO: 12 - protein, 119 aa, synthetic construct
  source 1..119: note = 4-C08 VH
DVQLVESGGGLVQPGGSLRLSCAVSGFSLSSYDMNWYRQGPGKEREWVANIHSSGGYPDYADAVKGRFTISRDNAKNMVYLQMNSLKPEDTAVYYCNLPPSRRWYKDYWGQGTQVTVSS

SEQ ID NO: 13 - protein, 8 aa, synthetic construct
  source 1..8: note = 4-E04 CDR1
EMISSTYI

SEQ ID NO: 14 - protein, 8 aa, synthetic construct
  source 1..8: note = 4-E04 CDR2
ISGDGVTH

SEQ ID NO: 15 - protein, 8 aa, synthetic construct
  source 1..8: note = 4-E04 CDR3
NAAGRRNH

SEQ ID NO: 16 - protein, 114 aa, synthetic construct
  source 1..114: note = 4-E04 VH
AVQLVESGGGLVQPGGSLSLSCAASEMISSTYIMGWYRRSPGKERELVAVISGDGVTHYGDFVKGRFAISRDNVKNAVYLKMNFLTPEDTAVYYCNAAGRRNHWGQGTQVTVSS

SEQ ID NO: 17 - protein, 8 aa, synthetic construct
  source 1..8: note = 4-C05 CDR1
GFTLDTYA

SEQ ID NO: 18 - protein, 8 aa, synthetic construct
  source 1..8: note = 4-C05 CDR2
ISSTDGST

SEQ ID NO: 19 - protein, 14 aa, synthetic construct
  source 1..14: note = 4-C05 CDR3
AAGPGTDCPLRFDY

SEQ ID NO: 20 - protein, 121 aa, synthetic construct
  source 1..121: note = 4-C05 VH
QVQLVESGGGLVQPGGSLRLSCAASGFTLDTYAIGWIRQAPGKEREGVSCISSTDGSTYYAASVKGRFTINRDNAKNTVYLQMNSLKPEDTAVYYCAAGPGTDCPLRFDYWGQGIQVTVSS

SEQ ID NO: 21 - protein, 8 aa, synthetic construct
  source 1..8: note = 5-C12 CDR1
GRTFSTDA

SEQ ID NO: 22 - protein, 8 aa, synthetic construct
  source 1..8: note = 5-C12 CDR2
INWSGGST

SEQ ID NO: 23 - protein, 22 aa, synthetic construct
  source 1..22: note = 5-C12 CDR3
VADSLLALLDGSRGGPGTDSDS

SEQ ID NO: 24 - protein, 129 aa, synthetic construct
  source 1..129: note = 5-C12 VH
QVQLVESGGGLAQAGGSLRLSCAGSGRTFSTDAMGWFRQAPGKEREFVAAINWSGGSTYYADSVKGRFTISRDNAKNTVYLQMNSVKPEDTAVYYCVADSLLALLDGSRGGPGTDSDSWGQGTQVTVSS

SEQ ID NO: 25 - protein, 8 aa, synthetic construct
  source 1..8: note = 5-H3 CDR1
GFTLANYA

SEQ ID NO: 26 - protein, 8 aa, synthetic construct
  source 1..8: note = 5-H3 CDR2
ISRSDGDT

SEQ ID NO: 27 - protein, 14 aa, synthetic construct
  source 1..14: note = 5-H3 CDR3
RATEWCGVQDPHGY

SEQ ID NO: 28 - protein, 121 aa, synthetic construct
  source 1..121: note = 5-H3 VH
QVQLVESGGGLVQPGGSLRLSCVASGFTLANYAIGFYRRAPGKGREGVSCISRSDGDTYHVDSVKGRFTVSRDNAKNTAYLQMNSLVPEDTGVYYCRATEWCGVQDPHGYWGQGTQVTVSS

SEQ ID NO: 29 - protein, 346 aa, synthetic construct
  source 1..346: note = 4-A02-FC1
QVQLVESGGGLVQPGGSLSLSCTASETISSTYIMGWHRRSPGKERELVAVISGDGVTHYADFVKGRFVISRDNAKNAVYLKMNFLTPEDTAVYYCYAAGRWNHWGQGTQVTVSSEPKSSDKTHTCPPCPAPEFEGGPSVFLFPPKPKDTLMISRTPEVTCVVVDVSHEDPEVKFNWYVDGVEVHNAKTKPREEQYNSTYRVVSVLTVLHQDWLNGKEYKCKVSNKALPASIEKTISKAKGQPREPQVYTLPPSRDELTKNQVSLTCLVKGFYPSDIAVEWESNGQPENNYKTTPPVLDSDGSFFLYSKLTVDKSRWQQGNVFSCSVMHEALHNHYTQKSLSLSPGK

SEQ ID NO: 30 - protein, 346 aa, synthetic construct
  source 1..346: note = 4-A02-FCWT
QVQLVESGGGLVQPGGSLSLSCTASETISSTYIMGWHRRSPGKERELVAVISGDGVTHYADFVKGRFVISRDNAKNAVYLKMNFLTPEDTAVYYCYAAGRWNHWGQGTQVTVSSEPKSSDKTHTCPPCPAPELLGGPSVFLFPPKPKDTLMISRTPEVTCVVVDVSHEDPEVKFNWYVDGVEVHNAKTKPREEQYNSTYRVVSVLTVLHQDWLNGKEYKCKVSNKALPAPIEKTISKAKGQPREPQVYTLPPSREEMTKNQVSLTCLVKGFYPSDIAVEWESNGQPENNYKTTPPVLDSDGSFFLYSKLTVDKSRWQQGNVFSCSVMHEALHNHYTQKSLSLSPGK

SEQ ID NO: 31 - protein, 346 aa, synthetic construct
  source 1..346: note = 4-A02-FCLALAPG
QVQLVESGGGLVQPGGSLSLSCTASETISSTYIMGWHRRSPGKERELVAVISGDGVTHYADFVKGRFVISRDNAKNAVYLKMNFLTPEDTAVYYCYAAGRWNHWGQGTQVTVSSEPKSSDKTHTCPPCPAPEAAGGPSVFLFPPKPKDTLMISRTPEVTCVVVDVSHEDPEVKFNWYVDGVEVHNAKTKPREEQYNSTYRVVSVLTVLHQDWLNGKEYKCKVSNKALGAPIEKTISKAKGQPREPQVYTLPPSREEMTKNQVSLTCLVKGFYPSDIAVEWESNGQPENNYKTTPPVLDSDGSFFLYSKLTVDKSRWQQGNVFSCSVMHEALHNHYTQKSLSLSPGK

SEQ ID NO: 32 - protein, 198 aa, synthetic construct
  source 1..198: note = 4-A02-ABD
QVQLVESGGGLVQPGGSLSLSCTASETISSTYIMGWHRRSPGKERELVAVISGDGVTHYADFVKGRFVISRDNAKNAVYLKMNFLTPEDTAVYYCYAAGRWNHWGQGTQVTVSSGGGGSGGGGSGGGGSQHDEAVDANSLAEAKVLANRELDKYGVSDYYKNLINNAKTVEGVKALIDEILAALPAAACAAAHHHHHH

SEQ ID NO: 33 - protein, 346 aa, synthetic construct
  source 1..346: note = 4A02-HM7-FCWT
QVQLVESGGGLVQPGGSLRLSCTASETISSTYIMGWHRQAPGKGRELVAVISGDGVTHYADFVKGRFTISRDNAKNTVYLQMNFLRAEDTAVYYCYAAGRWNHWGQGTMVTVSSEPKSSDKTHTCPPCPAPELLGGPSVFLFPPKPKDTLMISRTPEVTCVVVDVSHEDPEVKFNWYVDGVEVHNAKTKPREEQYNSTYRVVSVLTVLHQDWLNGKEYKCKVSNKALPAPIEKTISKAKGQPREPQVYTLPPSREEMTKNQVSLTCLVKGFYPSDIAVEWESNGQPENNYKTTPPVLDSDGSFFLYSKLTVDKSRWQQGNVFSCSVMHEALHNHYTQKSLSLSPGK

SEQ ID NO: 34 - protein, 346 aa, synthetic construct
  source 1..346: note = 4A02-HM8-FCWT
QVQLVESGGGLVKPGGSLRLSCTASETISSTYIMGWHRQAPGKGRELVAVISGDGVTHYADFVKGRFTISRDNAKNTVYLQMNFLRAEDTAVYYCYAAGRWNHWGQGTMVTVSSEPKSSDKTHTCPPCPAPELLGGPSVFLFPPKPKDTLMISRTPEVTCVVVDVSHEDPEVKFNWYVDGVEVHNAKTKPREEQYNSTYRVVSVLTVLHQDWLNGKEYKCKVSNKALPAPIEKTISKAKGQPREPQVYTLPPSREEMTKNQVSLTCLVKGFYPSDIAVEWESNGQPENNYKTTPPVLDSDGSFFLYSKLTVDKSRWQQGNVFSCSVMHEALHNHYTQKSLSLSPGK

SEQ ID NO: 35 - protein, 346 aa, synthetic construct
  source 1..346: note = 4A02-HM9-FCWT
QVQLVESGGGLVQPGGSLRLSCTASETISSTYIMGWHRQAPGKGLELVAVISGDGVTHYADFVKGRFTISRDNAKNAVYLQMNFLRAEDTAVYYCYAAGRWNHWGQGTMVTVSSEPKSSDKTHTCPPCPAPELLGGPSVFLFPPKPKDTLMISRTPEVTCVVVDVSHEDPEVKFNWYVDGVEVHNAKTKPREEQYNSTYRVVSVLTVLHQDWLNGKEYKCKVSNKALPAPIEKTISKAKGQPREPQVYTLPPSREEMTKNQVSLTCLVKGFYPSDIAVEWESNGQPENNYKTTPPVLDSDGSFFLYSKLTVDKSRWQQGNVFSCSVMHEALHNHYTQKSLSLSPGK